European Patent Specification EP 3 814 513 B1, published April 9, 2025. Title: Optimized CLN5 Genes and Expression Cassettes and Their Use. Applicant: The University of North Carolina at Chapel Hill Lincoln University Gray, Steven James Palmer, David Mitchell, Nadia. The sequence listing filed with the application follows.

SEQUENCE LISTING (11 sequences)

SEQ ID NO: 1 - DNA, 1077 bp, Artificial
  human CLN5 ORF
atggcgcaggaggtggacactgcacagggggccgagatgagaagaggagccggagcagctagaggacgggccagctggtgttgggccttggcgctgctctggctggctgtggtgcctggctggtccagagtgtccgggattccctcgaggcgccattggcctgtgccatataagcgcttcgacttccggcctaagcccgacccgtactgccaggccaagtacaccttttgtcccaccggatcgcccatccctgtgatggagggcgacgatgacatcgaagtgttccgactgcaagcccccgtgtgggaattcaaatacggcgaccttctgggccacctgaagatcatgcatgacgccatcgggttccgctcgaccctgaccggaaagaactacaccatggagtggtacgaactgttccagctgggaaactgcaccttccctcaccttcggcctgaaatggatgcacctttctggtgcaaccaaggcgctgcctgcttctttgaggggatcgacgatgtgcactggaaggagaacggaaccctggtccaagtggccactatctccgggaacatgttcaaccagatggccaaatgggtgaagcaggataatgagactggcatctactatgaaacttggaacgtgaaagccagcccggagaagggtgccgaaacctggttcgattcctacgactgctccaagttcgtgctgcggaccttcaacaagctggccgagttcggtgccgagttcaagaacattgaaaccaactacactcgcattttcctctactcgggcgaacccacctacctgggaaacgaaactagcgtctttgggccgactggaaacaagactttggggctcgcgatcaagaggttctactaccctttcaagccgcaccttccgaccaaggaattcttgctgagcctgctgcagattttcgatgccgtgatcgtgcataagcagttctatctgttttacaatttcgaatactggttcctcccgatgaagttcccgttcattaagatcacctacgaggaaatcccactcccgatccgcaacaagaccctgtccggtctgtaa

SEQ ID NO: 2 - DNA, 1089 bp, Artificial
  ovine CLN5 ORF
atggcacaagcaggaggagcaggggcaggagcttggggaaggagaggagcaggagctggagcgggccctgagcgggccccttggcgctgggccccggccctgctgtggctcgcggcggctactgccgctgccgccgccgccggggacccgtcccggagacagtggccggtgccatacaagcgcttcagctttcggcccgagccggacccgtactgtcaggccaagtacaccttctgcccaaccggctcccctatcccggtcatgaaggacgacgacgtcattgaagtgttcaggctccaagcccccgtgtgggagttcaaatacggagatctgcttggtcacttgaagattatgcacgatgcgatcggctttcgctccaccctgaccgagaagaactacactatggagtggtacgaattgttccagctgggcaactgcactttcccccacctgaggcccgagatgaacgcgcctttctggtgtaaccagggtgcagcctgctttttcgagggcatcgacgacaaccattggaaggagaacggcaccctggtcctggtggccacaatcagcggcgggatgttcaacaagatggccaaatgggtgaagcaggacaacgagactggaatctattacgagacttggaccgtgcaagcctcacccaagaaggaggccgagaagtggttcgagtcctacgactgctcaaagttcgtgctgcgcacctacgaaaagctggccgaacttggagccgacttcaagaagatcgaaaccaactacacccgcatctttctgtattcgggcgaacccacgtacctgggaaacgaaacctccgtgttcggccctaccgggaacaagactcttgctctcgccatcaagaagttctactacccgttcaagccgcacctgtcgaccaaggaattcctcctgagcctgctgcagatctttgatgcggtggtcattcaccgggaattctatctgttctacaatttcgagtactggttcctccctatgaaatccccattcattaagatcacttacgaagaaattccgctccccaatcgcaaaaaccggaccctgtccggtctgtgataa

SEQ ID NO: 3 - DNA, 306 bp, Artificial
  chicken beta actin promoter
tacgtattagtcatcgctattaccatggtcgaggtgagccccacgttctgcttcactctccccatctcccccccctccccacccccaattttgtatttatttattttttaattattttgtgcagcgatgggggcggggggggggggggggcgcgcgccaggcggggcggggcggggcgaggggcggggcggggcgaggcggagaggtgcggcggcagccaatcagagcggcgcgctccgaaagtttccttttatggcgaggcggcggcggcggcggccctataaaaagcgaagcgcgcggcgggcg

SEQ ID NO: 4 - DNA, 137 bp, Artificial
  Chimeric intron
ggagtcgctgcgacgctgccttcgccccgtgccccgctccgccgccgcctcgcgccgcccgccccggctctgactgaccgcgttactcccacaggtgagcgggcgggacggcccttctcctccgggctgtaattagc

SEQ ID NO: 5 - DNA, 1881 bp, Artificial
  CAGGS promoter
gatctgaattcggatcttcaatattggccattagccatattattcattggttatatagcataaatcaatattggatattggccattgcatacgttgtatctatatcataatatgtacatttatattggctcatgtccaatatgaccgccatgttggcattgattattgactagttattaatagtaatcaattacggggtcattagttcatagcccatatatggagttccgcgttacataacttacggtaaatggcccgcctggctgaccgcccaacgacccccgcccattgacgtcaataatgacgtatgttcccatagtaacgccaatagggactttccattgacgtcaatgggtggagtatttacggtaaactgcccacttggcagtacatcaagtgtatcatatgccaagtccgccccctattgacgtcaatgacggtaaatggcccgcctggcattatgcccagtacatgaccttacgggactttcctacttggcagtacatctacgtattagtcatcgctattaccatggtcgaggtgagccccacgttctgcttcactctccccatctcccccccctccccacccccaattttgtatttatttattttttaattattttgtgcagcgatgggggcggggggggggggggggcgcgcgccaggcggggcggggcggggcgaggggcggggcggggcgaggcggagaggtgcggcggcagccaatcagagcggcgcgctccgaaagtttccttttatggcgaggcggcggcggcggcggccctataaaaagcgaagcgcgcggcgggcgggagtcgctgcgacgctgccttcgccccgtgccccgctccgccgccgcctcgcgccgcccgccccggctctgactgaccgcgttactcccacaggtgagcgggcgggacggcccttctcctccgggctgtaattagcgcttggtttaatgacggcttgtttcttttctgtggctgcgtgaaagccttgaggggctccgggagggccctttgtgcgggggggagcggctcggggggtgcgtgcgtgtgtgtgtgcgtggggagcgccgcgtgcggcccgcgctgcccggcggctgtgagcgctgcgggcgcggcgcggggctttgtgcgctccgcagtgtgcgcgaggggagcgcggccgggggcggtgccccgcggtgcggggggggctgcgaggggaacaaaggctgcgtgcggggtgtgtgcgtgggggggtgagcagggggtatgggcgcggcggtcgggctgtaacccccccctgcacccccctccccgagttgctgagcacggcccggcttcgggtgcggggctccgtacggggcgtggcgcggggctcgccgtgccgggcggggggtggcggcaggtgggggtgccgggcggggcggggccgcctcgggccggggagggctcgggggaggggcgcggcggcccccggagcgccggcggctgtcgaggcgcggcgagccgcagccattgccttttatggtaatcgtgcgagagggcgcagggacttactttgtcccaaatctgtgcggagccgaaatctgggaggcgccgccgcaccccctctagcgggcgcggggcgaagcggtgcggcgccggcaggaaggaaatgggcggggagggccttcgtgcgtcgccgcgccgccgtccccttctccctctccagcctcggggctgtccgcggggggacggctgccttcgggggggacggggcagggcggggttcggcttctggcgtgtgaccggcggctctagagcctctgctaaccatgttcatgccttcttctttttcctacagctcctgggcaacgtgctggttattgtgctgtctcatcattttggcaaag

SEQ ID NO: 6 - DNA, 256 bp, Artificial
  CMV enhancer
tacataacttacggtaaatggcccgcctggctgaccgcccaacgacccccgcccattgacgtcaatagtaacgccaatagggactttccattgacgtcaatgggtggagtatttacggtaaactgcccacttggcagtacatcaagtgtatcatatgccaagtacgccccctattgacgtcaatgacggtaaatggcccgcctggcattgtgcccagtacatgaccttatgggactttcctacttggcagtacatc

SEQ ID NO: 7 - DNA, 48 bp, Artificial
  SpA
aataaagagctcagatgcatcgatcagagtgtgttggttttttgtgtg

SEQ ID NO: 8 - DNA, 143 bp, Artificial
  SV40pA
agacatgataagatacattgatgagtttggacaaaccacaactagaatgcagtgaaaaaaatgctttatttgtgaaatttgtgatgctattgctttatttgtaaccattataagctgcaataaacaagttaacaacaacaatt

SEQ ID NO: 9 - DNA, 254 bp, Artificial
  BGHpA
ctcgactgtgccttctagttgccagccatctgttgtttgcccctcccccgtgccttccttgaccctggaaggtgccactcccactgtcctttcctaataaaatgaggaaattgcatcgcattgtctgagtaggtgtcattctattctggggggtggggtggggcaggacagcaagggggaggattgggaagacaacagcaggcatgctggggatgcggtgggctctatggcttctgaggcggaaagaaccagct

SEQ ID NO: 10 - DNA, 2176 bp, Artificial
  Human CLN5 cassette
tacataacttacggtaaatggcccgcctggctgaccgcccaacgacccccgcccattgacgtcaataatgacgtatgttcccatagtaacgccaatagggactttccattgacgtcaatgggtggagtatttacggtaaactgcccacttggcagtacatcaagtgtatcatatgccaagtacgccccctattgacgtcaatgacggtaaatggcccgcctggcattatgcccagtacatgaccttatgggactttcctacttggcagtacatctacgtattagtcatcgctattaccatggtcgaggtgagccccacgttctgcttcactctccccatctcccccccctccccacccccaattttgtatttatttattttttaattattttgtgcagcgatgggggcggggggggggggggggcgcgcgccaggcggggcggggcggggcgaggggcggggcggggcgaggcggagaggtgcggcggcagccaatcagagcggcgcgctccgaaagtttccttttatggcgaggcggcggcggcggcggccctataaaaagcgaagcgcgcggcgggcgggagtcgctgcgacgctgccttcgccccgtgccccgctccgccgccgcctcgcgccgcccgccccggctctgactgaccgcgttactcccacaggtgagcgggcgggacggcccttctcctccgggctgtaattagctgagcaagaggtaagggtttaagggatggttggttggtggggtattaatgtttaattacctggagcacctgcctgaaatcactttttttcaggttggaccggtcgccaccatggcgcaggaggtggacactgcacagggggccgagatgagaagaggagccggagcagctagaggacgggccagctggtgttgggccttggcgctgctctggctggctgtggtgcctggctggtccagagtgtccgggattccctcgaggcgccattggcctgtgccatataagcgcttcgacttccggcctaagcccgacccgtactgccaggccaagtacaccttttgtcccaccggatcgcccatccctgtgatggagggcgacgatgacatcgaagtgttccgactgcaagcccccgtgtgggaattcaaatacggcgaccttctgggccacctgaagatcatgcatgacgccatcgggttccgctcgaccctgaccggaaagaactacaccatggagtggtacgaactgttccagctgggaaactgcaccttccctcaccttcggcctgaaatggatgcacctttctggtgcaaccaaggcgctgcctgcttctttgaggggatcgacgatgtgcactggaaggagaacggaaccctggtccaagtggccactatctccgggaacatgttcaaccagatggccaaatgggtgaagcaggataatgagactggcatctactatgaaacttggaacgtgaaagccagcccggagaagggtgccgaaacctggttcgattcctacgactgctccaagttcgtgctgcggaccttcaacaagctggccgagttcggtgccgagttcaagaacattgaaaccaactacactcgcattttcctctactcgggcgaacccacctacctgggaaacgaaactagcgtctttgggccgactggaaacaagactttggggctcgcgatcaagaggttctactaccctttcaagccgcaccttccgaccaaggaattcttgctgagcctgctgcagattttcgatgccgtgatcgtgcataagcagttctatctgttttacaatttcgaatactggttcctcccgatgaagttcccgttcattaagatcacctacgaggaaatcccactcccgatccgcaacaagaccctgtccggtctgtaatagcggccgcgcggatccctcgactgtgccttctagttgccagccatctgttgtttgcccctcccccgtgccttccttgaccctggaaggtgccactcccactgtcctttcctaataaaatgaggaaattgcatcgcattgtctgagtaggtgtcattctattctggggggtggggtggggcaggacagcaagggggaggattgggaagacaacagcaggcatgctggggatgcggtgggctctatggcttctgaggcggaaagaaccagct

SEQ ID NO: 11 - DNA, 2185 bp, Artificial
  Ovine CLN5 cassette
tacataacttacggtaaatggcccgcctggctgaccgcccaacgacccccgcccattgacgtcaataatgacgtatgttcccatagtaacgccaatagggactttccattgacgtcaatgggtggagtatttacggtaaactgcccacttggcagtacatcaagtgtatcatatgccaagtacgccccctattgacgtcaatgacggtaaatggcccgcctggcattatgcccagtacatgaccttatgggactttcctacttggcagtacatctacgtattagtcatcgctattaccatggtcgaggtgagccccacgttctgcttcactctccccatctcccccccctccccacccccaattttgtatttatttattttttaattattttgtgcagcgatgggggcggggggggggggggggcgcgcgccaggcggggcggggcggggcgaggggcggggcggggcgaggcggagaggtgcggcggcagccaatcagagcggcgcgctccgaaagtttccttttatggcgaggcggcggcggcggcggccctataaaaagcgaagcgcgcggcgggcgggagtcgctgcgacgctgccttcgccccgtgccccgctccgccgccgcctcgcgccgcccgccccggctctgactgaccgcgttactcccacaggtgagcgggcgggacggcccttctcctccgggctgtaattagctgagcaagaggtaagggtttaagggatggttggttggtggggtattaatgtttaattacctggagcacctgcctgaaatcactttttttcaggttggaccggtcgccaccatggcacaagcaggaggagcaggggcaggagcttggggaaggagaggagcaggagctggagcgggccctgagcgggccccttggcgctgggccccggccctgctgtggctcgcggcggctactgccgctgccgccgccgccggggacccgtcccggagacagtggccggtgccatacaagcgcttcagctttcggcccgagccggacccgtactgtcaggccaagtacaccttctgcccaaccggctcccctatcccggtcatgaaggacgacgacgtcattgaagtgttcaggctccaagcccccgtgtgggagttcaaatacggagatctgcttggtcacttgaagattatgcacgatgcgatcggctttcgctccaccctgaccgagaagaactacactatggagtggtacgaattgttccagctgggcaactgcactttcccccacctgaggcccgagatgaacgcgcctttctggtgtaaccagggtgcagcctgctttttcgagggcatcgacgacaaccattggaaggagaacggcaccctggtcctggtggccacaatcagcggcgggatgttcaacaagatggccaaatgggtgaagcaggacaacgagactggaatctattacgagacttggaccgtgcaagcctcacccaagaaggaggccgagaagtggttcgagtcctacgactgctcaaagttcgtgctgcgcacctacgaaaagctggccgaacttggagccgacttcaagaagatcgaaaccaactacacccgcatctttctgtattcgggcgaacccacgtacctgggaaacgaaacctccgtgttcggccctaccgggaacaagactcttgctctcgccatcaagaagttctactacccgttcaagccgcacctgtcgaccaaggaattcctcctgagcctgctgcagatctttgatgcggtggtcattcaccgggaattctatctgttctacaatttcgagtactggttcctccctatgaaatccccattcattaagatcacttacgaagaaattccgctccccaatcgcaaaaaccggaccctgtccggtctgtgataacggccgcgcggatccctcgactgtgccttctagttgccagccatctgttgtttgcccctcccccgtgccttccttgaccctggaaggtgccactcccactgtcctttcctaataaaatgaggaaattgcatcgcattgtctgagtaggtgtcattctattctggggggtggggtggggcaggacagcaagggggaggattgggaagacaacagcaggcatgctggggatgcggtgggctctatggcttctgaggcggaaagaaccagct